European Patent Application EP 4 755 919 A1, published June 10, 2026. Title: 抗Trop2抗体、包含所述抗体的缀合物及其应用. Applicant: 上海洛启生物医药技术有限公司. The sequence listing filed with the application follows.

SEQUENCE LISTING (36 sequences)

SEQ ID NO: 1 - protein, 128 aa, synthetic construct
  source 1..128: note = Trop2 Nb1
QVQLQESGGGSVQAGGSLRLSCAASGFTFSRACMGWFRQASGKEREGVAQVYTGGGSTSYADSVKGRFTISQDNAKNTLYLQMNSLKPEDTAVYYCAVGQPYGACYYSDLAPADFSYWGQGTQVTVSS

SEQ ID NO: 2 - protein, 25 aa, synthetic construct
  source 1..25: note = Trop2 Nb1 FR1
QVQLQESGGGSVQAGGSLRLSCAAS

SEQ ID NO: 3 - protein, 15 aa, synthetic construct
  source 1..15: note = Trop2 Nb1 FR2
WFRQASGKEREGVAQ

SEQ ID NO: 4 - protein, 38 aa, synthetic construct
  source 1..38: note = Trop2 Nb1 FR3
SYADSVKGRFTISQDNAKNTLYLQMNSLKPEDTAVYYC

SEQ ID NO: 5 - protein, 11 aa, synthetic construct
  source 1..11: note = Trop2 Nb1 FR4
WGQGTQVTVSS

SEQ ID NO: 6 - protein, 10 aa, synthetic construct
  source 1..10: note = Trop2 Nb1 CDR1
GFTFSRACMG

SEQ ID NO: 7 - protein, 8 aa, synthetic construct
  source 1..8: note = Trop2 Nb1 CDR2
VYTGGGST

SEQ ID NO: 8 - protein, 21 aa, synthetic construct
  source 1..21: note = Trop2 Nb1 CDR3
AVGQPYGACYYSDLAPADFSY

SEQ ID NO: 9 - protein, 128 aa, synthetic construct
  source 1..128: note = Trop2 HuNb1
EVQLLESGGGLVQPGGSLRLSCAASGFTFSRACMGWFRQASGKGLEGVAQVYTGGGSTSYADSVKGRFTISQDNAKNTLYLQMNSLKPEDTAVYYCAVGQPYGACYYSDLAPADFSYWGQGTLVTVSS

SEQ ID NO: 10 - protein, 25 aa, synthetic construct
  source 1..25: note = Trop2 HuNb1 FR1
EVQLLESGGGLVQPGGSLRLSCAAS

SEQ ID NO: 11 - protein, 15 aa, synthetic construct
  source 1..15: note = Trop2 HuNb1 FR2
WFRQASGKGLEGVAQ

SEQ ID NO: 12 - protein, 38 aa, synthetic construct; identical to SEQ ID NO: 4
  source 1..38: note = Trop2 HuNb1 FR3

SEQ ID NO: 13 - protein, 11 aa, synthetic construct
  source 1..11: note = Trop2 HuNb1 FR4
WGQGTLVTVSS

SEQ ID NO: 14 - protein, 125 aa, synthetic construct
  source 1..125: note = Trop2 HuNb2
EVQLLESGGGLVQPGGSLRLSCVDSGSTYSRRYMGWFRRAPGKGLEGVSVISPYGDSTYYADSVKDRFTISRDNAKNTVYLQMNSLKPEDTAMYYCAASWPYQTASLDAMDFTDWGQGTLVTVSS

SEQ ID NO: 15 - protein, 118 aa, synthetic construct
  source 1..118: note = Alb Nb1
EVQLQESGGGLVEPGGSLRLSCVASGFTFQHYAMSWVRQAPGKGLEWVSSISLVGGGTSYADSVKGRFTMSRDNAKNTLYLQLNSLKSEDTAMYYCVRGWHPDVPRPLGQGTLVTVSS

SEQ ID NO: 16 - protein, 266 aa, synthetic construct
  source 1..266: note = HuNb1-Alb Nb1
EVQLLESGGGLVQPGGSLRLSCAASGFTFSRACMGWFRQASGKGLEGVAQVYTGGGSTSYADSVKGRFTISQDNAKNTLYLQMNSLKPEDTAVYYCAVGQPYGACYYSDLAPADFSYWGQGTLVTVSSGGGGSGGGGSGGGGSGGGGSEVQLQESGGGLVEPGGSLRLSCVASGFTFQHYAMSWVRQAPGKGLEWVSSISLVGGGTSYADSVKGRFTMSRDNAKNTLYLQLNSLKSEDTAMYYCVRGWHPDVPRPLGQGTLVTVSS

SEQ ID NO: 17 - protein, 269 aa, synthetic construct
  source 1..269: note = HuNb1-Alb Nb1-GGC
EVQLLESGGGLVQPGGSLRLSCAASGFTFSRACMGWFRQASGKGLEGVAQVYTGGGSTSYADSVKGRFTISQDNAKNTLYLQMNSLKPEDTAVYYCAVGQPYGACYYSDLAPADFSYWGQGTLVTVSSGGGGSGGGGSGGGGSGGGGSEVQLQESGGGLVEPGGSLRLSCVASGFTFQHYAMSWVRQAPGKGLEWVSSISLVGGGTSYADSVKGRFTMSRDNAKNTLYLQLNSLKSEDTAMYYCVRGWHPDVPRPLGQGTLVTVSSGGC

SEQ ID NO: 18 - DNA, 384 bp, synthetic construct
  source 1..384: mol_type = other DNA; note = Trop2 Nb1
caggttcagctgcaggaatctggtggtggttctgttcaggcgggtggttctctgcgtctgtcttgcgcggcgtctggtttcaccttctctcgtgcgtgcatgggttggttccgtcaggcgtctggtaaagaacgtgaaggtgttgcgcaggtttacaccggtggtggttctacctcttacgcggactctgttaaaggtcgtttcaccatctctcaggacaacgcgaaaaacaccctgtacctgcagatgaactctctgaaaccggaagacaccgcggtttactactgcgcggttggtcagccgtacggtgcgtgctactactctgacctggcgccggcggacttctcttactggggtcagggtacccaggttaccgtttcttct

SEQ ID NO: 19 - DNA, 384 bp, synthetic construct
  source 1..384: mol_type = other DNA; note = Trop2 HuNb1
gaggtccagctgctggagagcggaggcggactcgtccagcctggcggctccctccggctctcctgtgccgcttctggatttacatttagcagggcttgtatgggatggttcaggcaggcttcagggaaagggttggagggtgttgcccaggtttataccggagggggcagcacttcctacgccgattcagtcaaaggcaggtttaccatctcccaggataatgctaagaataccctgtatctccagatgaacagtttgaaacccgaggacacagctgtgtactactgtgctgtggggcagccctacggagcatgctattatagcgatctcgccccagcagacttttcatactgggggcaggggaccctcgttacagtttcctct

SEQ ID NO: 20 - DNA, 375 bp, synthetic construct
  source 1..375: mol_type = other DNA; note = Trop2 HuNb2
gaagtgcagctgctggagagcggaggaggactggttcagcctggaggaagcctgagactgagctgcgtggacagcggaagcacatacagcagaagatacatgggatggttcagaagagcacctggaaaaggcctggagggggtgtctgtgatcagcccttatggagacagcacctactacgccgatagcgtgaaggacagattcaccataagccgggacaacgccaagaacacagtgtacctgcaaatgaacagcctgaagcccgaagatactgctatgtactactgcgccgccagctggccttaccagacagcttcactggacgctatggattttaccgattggggccaggggaccctggttacagtctctagc

SEQ ID NO: 21 - DNA, 354 bp, synthetic construct
  source 1..354: mol_type = other DNA; note = Alb Nb1
gaggttcagttgcaggaaagtggcggtgggctggtggagcccggaggttccctccgcttgagttgcgtcgcctctggttttacctttcagcactatgctatgtcatgggttcgccaggccccagggaaggggctggagtgggtcagttctatttccctggtcggtggcggaacatcctatgcagattctgtgaaggggcgctttacaatgtcccgcgacaatgccaagaacactttgtacctgcagctcaactctctgaagtccgaagatacagccatgtattactgcgtgcgtggatggcatccagacgtgcctagacccctcggccagggtacattggtgacagtctccagc

SEQ ID NO: 22 - DNA, 798 bp, synthetic construct
  source 1..798: mol_type = other DNA; note = HuNb1-Alb Nb1
gaggtccagctgctggagagcggaggcggactcgtccagcctggcggctccctccggctctcctgtgccgcttctggatttacatttagcagggcttgtatgggatggttcaggcaggcttcagggaaagggttggagggtgttgcccaggtttataccggagggggcagcacttcctacgccgattcagtcaaaggcaggtttaccatctcccaggataatgctaagaataccctgtatctccagatgaacagtttgaaacccgaggacacagctgtgtactactgtgctgtggggcagccctacggagcatgctattatagcgatctcgccccagcagacttttcatactgggggcaggggaccctcgttacagtttcctctggtggcggagggtctggtggtggaggatcagggggtggaggttcaggaggcgggggaagtgaggttcagttgcaggaaagtggcggtgggctggtggagcccggaggttccctccgcttgagttgcgtcgcctctggttttacctttcagcactatgctatgtcatgggttcgccaggccccagggaaggggctggagtgggtcagttctatttccctggtcggtggcggaacatcctatgcagattctgtgaaggggcgctttacaatgtcccgcgacaatgccaagaacactttgtacctgcagctcaactctctgaagtccgaagatacagccatgtattactgcgtgcgtggatggcatccagacgtgcctagacccctcggccagggtacattggtgacagtctccagc

SEQ ID NO: 23 - DNA, 807 bp, synthetic construct
  source 1..807: mol_type = other DNA; note = HuNb1-Alb Nb1-GGC
gaggtccagctgctggagagcggaggcggactcgtccagcctggcggctccctccggctctcctgtgccgcttctggatttacatttagcagggcttgtatgggatggttcaggcaggcttcagggaaagggttggagggtgttgcccaggtttataccggagggggcagcacttcctacgccgattcagtcaaaggcaggtttaccatctcccaggataatgctaagaataccctgtatctccagatgaacagtttgaaacccgaggacacagctgtgtactactgtgctgtggggcagccctacggagcatgctattatagcgatctcgccccagcagacttttcatactgggggcaggggaccctcgttacagtttcctctggtggcggagggtctggtggtggaggatcagggggtggaggttcaggaggcgggggaagtgaggttcagttgcaggaaagtggcggtgggctggtggagcccggaggttccctccgcttgagttgcgtcgcctctggttttacctttcagcactatgctatgtcatgggttcgccaggccccagggaaggggctggagtgggtcagttctatttccctggtcggtggcggaacatcctatgcagattctgtgaaggggcgctttacaatgtcccgcgacaatgccaagaacactttgtacctgcagctcaactctctgaagtccgaagatacagccatgtattactgcgtgcgtggatggcatccagacgtgcctagacccctcggccagggtacattggtgacagtctccagcgggggctgc

SEQ ID NO: 24 - protein, 10 aa, synthetic construct
  source 1..10: note = Alb Nb1 CDR1
GFTFQHYAMS

SEQ ID NO: 25 - protein, 8 aa, synthetic construct
  source 1..8: note = Alb Nb1 CDR2
ISLVGGGT

SEQ ID NO: 26 - protein, 11 aa, synthetic construct
  source 1..11: note = Alb Nb1 CDR3
VRGWHPDVPRP

SEQ ID NO: 27 - protein, 118 aa, synthetic construct
  source 1..118: note = HuNb3-11
EVQLQESGGGLVEPGGSLRLSCVASGFTFQHYAMSWVRQAPGKGLEWVSSISMVGGGTSYADSVKGRFTMSRDNAKNTLYLQLNSLKSEDTAMYYCVRGWHPDVPRPLGQGTLVTVSS

SEQ ID NO: 28 - protein, 8 aa, synthetic construct
  source 1..8: note = HuNb3-11 CDR1
ISMVGGGT

SEQ ID NO: 29 - protein, 8 aa, synthetic construct
  source 1..8: note = Alb Nb2 CDR2
ISVVGGGT

SEQ ID NO: 30 - protein, 8 aa, synthetic construct
  source 1..8: note = Alb Nb3 CDR2
ISIVGGGT

SEQ ID NO: 31 - protein, 8 aa, synthetic construct
  source 1..8: note = Alb Nb4 CDR2
ISTVGGGT

SEQ ID NO: 32 - protein, 8 aa, synthetic construct
  source 1..8: note = Alb Nb5 CDR2
ISGVGGGT

SEQ ID NO: 33 - protein, 8 aa, synthetic construct
  source 1..8: note = Alb Nb6 CDR2
ISYVGGGT

SEQ ID NO: 34 - protein, 118 aa, synthetic construct
  source 1..118: note = Alb Nb2
EVQLQESGGGLVEPGGSLRLSCVASGFTFQHYAMSWVRQAPGKGLEWVSSISVVGGGTSYADSVKGRFTMSRDNAKNTLYLQLNSLKSEDTAMYYCVRGWHPDVPRPLGQGTLVTVSS

SEQ ID NO: 35 - protein, 118 aa, synthetic construct
  source 1..118: note = Alb Nb3
EVQLQESGGGLVEPGGSLRLSCVASGFTFQHYAMSWVRQAPGKGLEWVSSISIVGGGTSYADSVKGRFTMSRDNAKNTLYLQLNSLKSEDTAMYYCVRGWHPDVPRPLGQGTLVTVSS

SEQ ID NO: 36 - protein, 118 aa, synthetic construct
  source 1..118: note = Alb Nb4
EVQLQESGGGLVEPGGSLRLSCVASGFTFQHYAMSWVRQAPGKGLEWVSSISTVGGGTSYADSVKGRFTMSRDNAKNTLYLQLNSLKSEDTAMYYCVRGWHPDVPRPLGQGTLVTVSS